European Patent Application EP 4 559 925 A1, published May 28, 2025. Title: METHOD FOR PRODUCING OLIGONUCLEOTIDE. Applicant: 住友化学株式会社. The sequence listing filed with the application follows.

SEQUENCE LISTING (4 sequences)

SEQ ID NO: 1 - RNA, 21 nt, synthetic construct
  source 1..21: mol_type = other RNA
  modified_base 7: mod_base = um
  modified_base 17: mod_base = um
  modified_base 20..21: mod_base = OTHER; note = thymidine
atggaanactcttggtnacnn

SEQ ID NO: 2 - RNA, 21 nt, synthetic construct
  source 1..21: mol_type = other RNA
  modified_base 2: mod_base = um
  modified_base 5..6: mod_base = cm
  modified_base 12: mod_base = um
  modified_base 14..15: mod_base = um
  modified_base 16..17: mod_base = cm
  modified_base 19: mod_base = um
  modified_base 20..21: mod_base = OTHER; note = thymidine
gnaannaagagnannnnannn

SEQ ID NO: 3 - RNA, 113 nt, synthetic construct
  source 1..113: mol_type = other RNA
  modified_base 1: mod_base = OTHER; note = 2'-O-methyladenosine
  modified_base 2: mod_base = gm
  modified_base 3: mod_base = um
  modified_base 110..112: mod_base = um
  misc_feature 1..4: note = phosphorothioate modification
  misc_feature 110..113: note = phosphorothioate modification
nnncctcatctccctcaagcgtttaagagctatgctggtaacagcatagcaagtttaaataaggctagtccgttatcaacttgaaaaagtggcaccgagtcggtgctttnnnt

SEQ ID NO: 4 - RNA, 25 nt, synthetic construct
  source 1..25: mol_type = other RNA
  modified_base 1..25: mod_base = um
ttttttttttttttttttttttttt